European Patent Application EP 4 265 637 A1, published October 25, 2023. Title: RESPIRATORY SYNCYTIAL VIRUS-SPECIFIC BINDING MOLECULE. Applicant: Trinomab Biotech Co., Ltd. The sequence listing filed with the application follows.

SEQUENCE LISTING (8 sequences)

SEQ ID NO: 1 - protein, 8 aa, Artificial Sequence
  synthetical protein
GYSFNNYY

SEQ ID NO: 2 - protein, 8 aa, Artificial Sequence
  synthetical protein
IYPGDSDT

SEQ ID NO: 3 - protein, 20 aa, Artificial Sequence
  synthetical protein
VRMDTVTTGAGVGFNWFFDL

SEQ ID NO: 4 - protein, 6 aa, Artificial Sequence
  synthetical protein
QSVTSY

SEQ ID NO: 5 - protein, 3 aa, Artificial Sequence
  synthetical protein
GAS

SEQ ID NO: 6 - protein, 10 aa, Artificial Sequence
  synthetical protein
QQYNDWPAIT

SEQ ID NO: 7 - protein, 127 aa, Artificial Sequence
  synthetical protein
QVQLVQSGAEVKKPGESLKISCQGSGYSFNNYYIGWVRQMPGKGLEWMVIIYPGDSDTKYSPSFQGQVTVSADRSINTAYLQWSSLRASDTAVYYCVRMDTVTTGAGVGFNWFFDLWGRGTLVTVSS

SEQ ID NO: 8 - protein, 108 aa, Artificial Sequence
  synthetical protein
EIVLTQSPATLSVSPGERATLSCRASQSVTSYLAWYQQKPGQAPRLLIYGASSRATGVPARFSGSGSETEFTLTISSLQSEDFAVYYCQQYNDWPAITFGQGTRLENK